European Patent Specification EP 3 934 757 B1, published February 22, 2023. Title: 2'3'-CYCLIC DINUCLEOTIDES AND PRODRUGS THEREOF. Applicant: Birkus, Gabriel Pav, Ondrej Kostov, Ondrej Brehova, Petra Kaiser, Martin Maxmilian. Application Not Yet Assigned. The sequence listing filed with the application follows.

SEQUENCE LISTING (10 sequences)

SEQ ID NO: 1 - DNA, 75 bp, Artificial Sequence
  Synthetic construct
aaagatcttggaaagtgaaaccttggaaaacgaaactggacaaagggaaactgcagaaactgaaacaaagcttaa

SEQ ID NO: 2 - DNA, 75 bp, Artificial Sequence
  Synthetic construct
ttaagctttgtttcagtttctgcagtttccctttgtccagtttcgttttccaaggtttcactttccaagatcttt

SEQ ID NO: 3 - DNA, 20 bp, Artificial Sequence
  Synthetic construct
tgcttgctcaactctacgtc

SEQ ID NO: 4 - DNA, 20 bp, Artificial Sequence
  Synthetic construct
gtggtttgtccaaactcatc

SEQ ID NO: 5 - DNA, 31 bp, Artificial Sequence
  Synthetic construct
gtgggatccgccccagctgagatctctgcag

SEQ ID NO: 6 - DNA, 38 bp, Artificial Sequence
  Synthetic construct
tatgcggccgcctattacacagtaacctcttccttttc

SEQ ID NO: 7 - DNA, 330 bp, Artificial Sequence
  Synthetic construct
atgtcgcatcaccatcatcatcaccaccatgggatgtcggactcagaagtcaatcaagaagctaagccagaggtcaagccagaagtcaagcctgagactcacatcaatttaaaggtgtccgatggatcttcagagatcttcttcaagatcaaaaagaccactcctttaagaaggctgatggaagcgttcgctaaaagacagggtaaggaaatggactccttaagattcttgtacgacggtattagaattcaagctgatcagacccctgaagatttggacatggaggataacgatattattgaggctcaccgcgaacagattggtggatcc

SEQ ID NO: 8 - protein, 110 aa, Artificial Sequence
  Synthetic construct
MSHHHHHHHHGMSDSEVNQEAKPEVKPEVKPETHINLKVSDGSSEIFFKIKKTTPLRRLMEAFAKRQGKEMDSLRFLYDGIRIQADQTPEDLDMEDNDIIEAHREQIGGS

SEQ ID NO: 9 - protein, 204 aa, Artificial Sequence
  Synthetic construct
APAEISAVCEKGNFNVAHGLAWSYYIGYLRLILPELQARIRTYNQHYNNLLRGAVSQRLYILLPLDCGVPDNLSMADPNIRFLDKLPQQTGDRAGIKDRVYSNSIYELLENGQRAGTCVLEYATPLQTLFAMSQYSQAGFSREDRLEQAKLFCRTLEDILADAPESQNNCRLIAYQEPADDSSFSLSQEVLRHLRQEEKEEVTV

SEQ ID NO: 10 - protein, 204 aa, Artificial Sequence
  Synthetic construct
APAEISAVCEKGNFNVAHGLAWSYYIGYLRLILPELQARIRTYNQHYNNLLRGAVSQRLYILLPLDCGVPDNLSMADPNIRFLDKLPQQTADRAGIKDRVYSNSIYELLENGQRAGTCVLEYATPLQTLFAMSQYSQAGFSREDRLEQAKLFCQTLEDILADAPESQNNCRLIAYQEPADDSSFSLSQEVLRHLRQEEKEEVTV